European Patent Specification EP 3 766 520 B1, published August 26, 2026. Title: Composition for Treating Hyperlipidemia Comprising Oxyntomodulin Derivative. Applicant: HANMI PHARM. CO., LTD. The sequence listing filed with the application follows.

SEQUENCE LISTING (53 sequences)

SEQ ID NO: 1 - protein, 37 aa, oxyntomodulin
HSQGTFTSDYSKYLDSRRAQDFVQWLMNTKRNRNNIA

SEQ ID NO: 2 - protein, 37 aa, oxyntomodulin derivative
  VARIANT (1): This "H" refers a derivative of histidine,  4-imidazoacetyl.
HSQGTFTSDYSKYLDEEAVRLFIEWLMNTKRNRNNIA

SEQ ID NO: 3 - protein, 39 aa, oxyntomodulin derivative
  VARIANT (1): This "H" refers a derivative of histidine,  4-imidazoacetyl.
HSQGTFTSDYSKYLDERRAQDFVAWLKNTGPSSGAPPPS

SEQ ID NO: 4 - protein, 39 aa, oxyntomodulin derivative
  VARIANT (1): This "H" refers a derivative of histidine,  4-imidazoacetyl.
HGQGTFTSDYSRYLEEEAVRLFIEWLKNGGPSSGAPPPS

SEQ ID NO: 5 - protein, 39 aa, oxyntomodulin derivative
  VARIANT (1): This "H" refers a derivative of histidine,  4-imidazoacetyl.
HGQGTFTSDYSRQMEEEAVRLFIEWLKNGGPSSGAPPPS

SEQ ID NO: 6 - protein, 42 aa, oxyntomodulin derivative
  VARIANT (1): This "H" refers a derivative of histidine,  4-imidazoacetyl.
HGEGTFTSDLSRQMEEEAVRLFIEWAAHSQGTFTSDYSKYLD

SEQ ID NO: 7 - protein, 30 aa, oxyntomodulin derivative
  VARIANT (1): This "H" refers a derivative of histidine,  4-imidazoacetyl.
HSQGTFTSDYSRYLDEEAVRLFIEWLMNTK

SEQ ID NO: 8 - protein, 29 aa, oxyntomodulin derivative
  VARIANT (1): This "H" refers a derivative of histidine,  4-imidazoacetyl.
HSQGTFTSDLSRQLEEEAVRLFIEWLMNK

SEQ ID NO: 9 - protein, 37 aa, oxyntomodulin derivative
  VARIANT (1): This "H" refers a derivative of histidine,  4-imidazoacetyl.
  VARIANT (20): Xaa = alpha-methyl-glutamic acid
HGQGTFTSDYSRYLDEEAVXLFIEWLMNTKRNRNNIA

SEQ ID NO: 10 - protein, 40 aa, oxyntomodulin derivative
  VARIANT (1): This "H" refers a derivative of histidine,  4-imidazoacetyl.
HSQGTFTSDYSRQMEEEAVRLFIEWLMNGGPSSGAPPPSK

SEQ ID NO: 11 - protein, 43 aa, oxyntomodulin derivative
  VARIANT (1): This "H" refers a derivative of histidine,  4-imidazoacetyl.
HGEGTFTSDLSRQMEEEAVRLFIEWAAHSQGTFTSDYSRYLDK

SEQ ID NO: 12 - protein, 38 aa, oxyntomodulin derivative
  VARIANT (1): This "H" refers a derivative of histidine,  4-imidazoacetyl.
HSQGTFTSDYSRYLDGGGHGEGTFTSDLSKQMEEEAVK

SEQ ID NO: 13 - protein, 30 aa, oxyntomodulin derivative
  VARIANT (1): This "H" refers a derivative of histidine,  4-imidazoacetyl.
  VARIANT (16): Xaa = alpha-methyl-glutamic acid
  VARIANT (20): Xaa = alpha-methyl-glutamic acid
HSQGTFTSDYSRYLDXEAVXLFIEWLMNTK

SEQ ID NO: 14 - protein, 37 aa, oxyntomodulin derivative
  VARIANT (1): This "H" refers a derivative of histidine,  4-imidazoacetyl.
  VARIANT (20): Xaa = alpha-methyl-glutamic acid
  VARIANT (24): Xaa = alpha-methyl-glutamic acid
HGQGTFTSDYSRYLDEEAVXLFIXWLMNTKRNRNNIA

SEQ ID NO: 15 - protein, 37 aa, oxyntomodulin derivative
  VARIANT (1): This "H" refers a derivative of histidine,  4-imidazoacetyl.
  VARIANT (24): Xaa = alpha-methyl-glutamic acid
HGQGTFTSDYSRYLDEEAVRLFIXWLMNTKRNRNNIA

SEQ ID NO: 16 - protein, 34 aa, oxyntomodulin derivative
  VARIANT (1): This "H" refers a derivative of histidine,  4-imidazoacetyl.
HSQGTFTSDLSRQLEGGGHSQGTFTSDLSRQLEK

SEQ ID NO: 17 - protein, 37 aa, oxyntomodulin derivative
  VARIANT (1): This "H" refers a derivative of histidine,  4-imidazoacetyl.
HSQGTFTSDYSRYLDEEAVRLFIEWIRNTKRNRNNIA

SEQ ID NO: 18 - protein, 40 aa, oxyntomodulin derivative
  VARIANT (1): This "H" refers a derivative of histidine,  4-imidazoacetyl.
HSQGTFTSDYSRYLDEEAVRLFIEWIRNGGPSSGAPPPSK

SEQ ID NO: 19 - protein, 37 aa, oxyntomodulin derivative
  VARIANT (1): This "H" refers a derivative of histidine,  4-imidazoacetyl.
HSQGTFTSDYSRYLDEEAVKLFIEWIRNTKRNRNNIA

SEQ ID NO: 20 - protein, 40 aa, oxyntomodulin derivative
  VARIANT (1): This "H" refers a derivative of histidine,  4-imidazoacetyl.
HSQGTFTSDYSRYLDEEAVKLFIEWIRNGGPSSGAPPPSK

SEQ ID NO: 21 - protein, 37 aa, oxyntomodulin derivative
  VARIANT (1): This "H" refers a derivative of histidine,  4-imidazoacetyl.
HSQGTFTSDYSRQLEEEAVRLFIEWVRNTKRNRNNIA

SEQ ID NO: 22 - protein, 30 aa, oxyntomodulin derivative
  VARIANT (1): This "H" refers a derivative of histidine,  desamino-histidyl.
HSQGTFTSDYSKYLDEKRAKEFVQWLMNTK

SEQ ID NO: 23 - protein, 29 aa, oxyntomodulin derivative
  VARIANT (2): Xaa = aminoisobutyric acid
HXQGTFTSDYSKYLDEKRAKEFVCWLMNT

SEQ ID NO: 24 - protein, 30 aa, oxyntomodulin derivative
  VARIANT (2): Xaa = aminoisobutyric acid
HXQGTFTSDYSKYLDEKRAKEFVQWLMNTC

SEQ ID NO: 25 - protein, 30 aa, oxyntomodulin derivative; identical to SEQ ID NO: 24
  VARIANT (2): Xaa = aminoisobutyric acid

SEQ ID NO: 26 - protein, 30 aa, oxyntomodulin derivative; identical to SEQ ID NO: 24
  VARIANT (2): Xaa = aminoisobutyric acid

SEQ ID NO: 27 - protein, 29 aa, Artificial Sequence
  oxyntomodulin derivative
  VARIANT (2): Xaa = aminoisobutyric acid
HXQGTFTSDYSKYLDEQAAKEFICWLMNT

SEQ ID NO: 28 - protein, 29 aa, oxyntomodulin derivative
  VARIANT (2): Xaa = aminoisobutyric acid
HXQGTFTSDYSKYLDEKRAKEFVQWLMNT

SEQ ID NO: 29 - protein, 37 aa, oxyntomodulin derivative; identical to SEQ ID NO: 1
  VARIANT (2): This "S" refers a variant of serine, d-serine.

SEQ ID NO: 30 - protein, 37 aa, oxyntomodulin derivative; identical to SEQ ID NO: 1
  VARIANT (1): This "H" refers a derivative of histidine,  4-imidazoacetyl

SEQ ID NO: 31 - protein, 37 aa, oxyntomodulin derivative; identical to SEQ ID NO: 1
  VARIANT (1): This "H" refers a derivative of histidine,  4-imidazoacetyl
  VARIANT (2): This "S" refers a variant of serine, d-serine.

SEQ ID NO: 32 - protein, 30 aa, Artificial Sequence; identical to SEQ ID NO: 24
  oxyntomodulin derivative
  VARIANT (1): This "H" refers a derivative of histidine,  4-imidazoacetyl.
  VARIANT (2): Xaa = aminoisobutyric acid

SEQ ID NO: 33 - protein, 30 aa, Artificial Sequence
  oxyntomodulin derivative
  VARIANT (2): Xaa = aminoisobutyric acid
HXQGTFTSDYAKYLDEKRAKEFVQWLMNTC

SEQ ID NO: 34 - protein, 30 aa, Artificial Sequence
  oxyntomodulin derivative
  VARIANT (2): Xaa = aminoisobutyric acid
YXQGTFTSDYSKYLDEKRAKEFVQWLMNTC

SEQ ID NO: 35 - protein, 8 aa, Artificial Sequence
  group R2
KRNRNNIA

SEQ ID NO: 36 - protein, 10 aa, Artificial Sequence
  group R2
GPSSGAPPPS

SEQ ID NO: 37 - protein, 11 aa, Artificial Sequence
  group R2
GPSSGAPPPSK

SEQ ID NO: 38 - protein, 15 aa, Artificial Sequence
  group R2
HSQGTFTSDYSKYLD

SEQ ID NO: 39 - protein, 16 aa, Artificial Sequence
  group R2
HSQGTFTSDYSRYLDK

SEQ ID NO: 40 - protein, 20 aa, Artificial Sequence
  group R2
HGEGTFTSDLSKQMEEEAVK

SEQ ID NO: 41 - protein, 28 aa, Artificial Sequence
  group A or B
SQGTFTSDYSKYLDSRRAQDFVQWLMNT

SEQ ID NO: 42 - protein, 28 aa, Artificial Sequence
  group A or B
SQGTFTSDYSKYLDEEAVRLFIEWLMNT

SEQ ID NO: 43 - protein, 28 aa, Artificial Sequence
  group A or B
SQGTFTSDYSKYLDERRAQDFVAWLKNT

SEQ ID NO: 44 - protein, 28 aa, Artificial Sequence
  group A or B
GQGTFTSDYSRYLEEEAVRLFIEWLKNG

SEQ ID NO: 45 - protein, 28 aa, Artificial Sequence
  group A or B
GQGTFTSDYSRQMEEEAVRLFIEWLKNG

SEQ ID NO: 46 - protein, 26 aa, Artificial Sequence
  group A or B
GEGTFTSDLSRQMEEEAVRLFIEWAA

SEQ ID NO: 47 - protein, 28 aa, Artificial Sequence
  group A or B
SQGTFTSDYSRQMEEEAVRLFIEWLMNG

SEQ ID NO: 48 - protein, 24 aa, Artificial Sequence
  group B
GEGTFTSDLSRQMEEEAVRLFIEW

SEQ ID NO: 49 - protein, 14 aa, Artificial Sequence
  group B
SQGTFTSDYSRYLD

SEQ ID NO: 50 - DNA, 30 bp, Artificial Sequence
  primer
cccggcccccgcggccgctattcgaaatac

SEQ ID NO: 51 - DNA, 33 bp, Artificial Sequence
  primer
gaacggtccggaggacgtcgactcttaagatag

SEQ ID NO: 52 - DNA, 34 bp, Artificial Sequence
  primer
cagcgacaccgaccgtccccccgtacttaaggcc

SEQ ID NO: 53 - DNA, 32 bp, Artificial Sequence
  primer
ctaaccgactctcggggaagactgagctcgcc